European Patent Application EP 4 410 972 A1, published August 7, 2024. Title: Modified benzalacetone synthase enzymes and uses thereof. Applicant: BGENE GENETICS. The sequence listing filed with the application follows.

SEQUENCE LISTING (29 sequences)

SEQ ID NO: 1 - protein, 384 aa, Rheum palmatum
MATEEMKKLATVMAIGTANPPNCYYQADFPDFYFRVTNSDHLINLKQKFKRLCENSRIEKRYLHVTEEILKENPNIAAYEATSLNVRHKMQVKGVAELGKEAALKAIKEWGQPKSKITHLIVCCLAGVDMPGADYQLTKLLDLDPSVKRFMFYHLGCYAGGTVLRLAKDIAENNKGARVLIVCSEMTTTCFRGPSETHLDSMIGQAILGDGAAAVIVGADPDLTVERPIFELVSTAQTIVPESHGAIEGHLLESGLSFHLYKTVPTLISNNIKTCLSDAFTPLNISDWNSLFWIAHPGGPAILDQVTAKVGLEKEKLKVTRQVLKDYGNMSSATVFFIMDEMRKKSLENGQATTGEGLEWGVLFGFGPGITVETVVLRSVPVIS

SEQ ID NO: 2 - protein, 384 aa, synthetic construct
MATEEMKKLATVMAIGTANPPNCYYQADFPDFYFRVTNSDHLINLKQKFKRLCENSRIEKRYLHVTEEILKENPNIAAYEATSLNVRHKMQVKGVAELGKEAALKAIKEWGQPKSKITHLIVCCLAGVDMPGADYQLTKLLDLDPSVKRFMFYHLGCYAGGTVLRLAKDIAENNKGARVLIVCSEMTTTCFRGPSETHLDSMIGQAILGDGAAAVIVGADPDLTVERPIFELVSTAQTIVPESHGAIEGHLLESGLSFHLYKTVPTLISNNIKTCLSDAFAPLNISDWNSLFWIAHPGGPAILDQVTAKVGLEKEKLKVTRQVLKDYGNMSSATVFFIMDEMRKKSLENGQATTGEGLEWGVLFGFGPGITVETVVLRSVPVIS

SEQ ID NO: 3 - DNA, 1155 bp, synthetic construct
  source 1..1155: mol_type = other DNA
atggcaactgaggagatgaagaaattggccaccgtgatggccattggcacggccaaccctccgaactgctactaccaggccgactttcccgacttctacttccgcgtcaccaacagcgaccacctcatcaacctcaagcaaaagttcaagcgcctttgtgaaaactcaaggattgagaagcgttaccttcatgtgaccgaagagattctcaaggaaaacccaaacattgctgcctacgaggcaacctcgttgaatgtaagacacaaaatgcaagtgaaaggagttgcagagcttgggaaagaggctgccctcaaggccatcaaagaatggggccaacccaagtccaagatcacacatctcatcgtgtgttgcctagccggcgttgacatgcccggcgcggattatcaactcactaagcttcttgaccttgacccttccgtcaagcgttttatgttttaccacctaggatgctacgctggtggcactgtccttcgccttgcaaaggacatagcggagaacaacaagggagctcgtgttctcatcgtttgctcagagatgacaacaacttgttttcgtgggccatctgaaacccatctggactccatgataggccaagcaatattaggcgatggggctgcagctgtcatagttggcgcagatccagacctaaccgttgagaggcccatattcgagttggtttccacagcccagactattgtacccgaatcccatggtgcaattgagggccacttgcttgaatctggactcagtttccatttgtacaagaccgttcctacactaatctctaacaacattaaaacttgcctttctgatgctttcgctcctctaaacattagcgattggaactctcttttctggatcgcacaccctggtggtcctgccatcctagaccaagttactgctaaggttggtcttgaaaaggagaaactcaaggtaactagacaagtgttgaaggactatggaaacatgtcgagtgctacggtgtttttcatcatggatgagatgaggaagaagtcactcgaaaacggtcaagcaaccactggagaagggctcgagtggggtgttttgtttgggttcgggcctggaatcaccgttgaaactgtagtgctacgcagtgtgcccgtaattagctag

SEQ ID NO: 4 - DNA, 5775 bp, synthetic construct
  source 1..5775: mol_type = other DNA
ctcgggccgtctcttgggcttgatcggccttcttgcgcatctcacgcgctcctgcggcggcctgtagggcaggctcatacccctgccgaaccgcttttgtcagccggtcggccacggcttccggcgtctcaacgcgctttgagattcccagcttttcggccaatccctgcggtgcataggcgcgtggctcgaccgcttgcgggctgatggtgacgtggcccactggtggccgctccagggcctcgtagaacgcctgaatgcgcgtgtgacgtgccttgctgccctcgatgccccgttgcagccctagatcggccacagcggccgcaaacgtggtctggtcgcgggtcatctgcgctttgttgccgatgaactccttggccgacagcctgccgtcctgcgtcagcggcaccacgaacgcggtcatgtgcgggctggtttcgtcacggtggatgctggccgtcacgatgcgatccgccccgtacttgtccgccagccacttgtgcgccttctcgaagaacgccgcctgctgttcttggctggccgacttccaccattccgggctggccgtcatgacgtactcgaccgccaacacagcgtccttgcgccgcttctctggcagcaactcgcgcagtcggcccatcgcttcatcggtgctgctggccgcccagtgctcgttctctggcgtcctgctggcgtcagcgttgggcgtctcgcgctcgcggtaggcgtgcttgagactggccgccacgttgcccattttcgccagcttcttgcatcgcatgatcgcgtatgccgccatgcctgcccctcccttttggtgtccaaccggctcgacgggggcagcgcaaggcggtgcctccggcgggccactcaatgcttgagtatactcactagactttgcttcgcaaagtcgtgaccgcctacggcggctgcggcgccctacgggcttgctctccgggcttcgccctgcgcggtcgctgcgctcccttgccagcccgtggatatgtggacgatggccgcgagcggccaccggctggctcgcttcgctcggcccgtggacaaccctgctggacaagctgatggacaggctgcgcctgcccacgagcttgaccacagggattgcccaccggctacccagccttcgaccacatacccaccggctccaactgcgcggcctgcggccttgccccatcaatttttttaattttctctggggaaaagcctccggcctgcggcctgcgcgcttcgcttgccggttggacaccaagtggaaggcgggtcaaggctcgcgcagcgaccgcgcagcggcttggccttgacgcgcctggaacgacccaagcctatgcgagtgggggcagtcgaaggcgaagcccgcccgcctgccccccgagcctcacggcggcgagtgcgggggttccaagggggcagcgccaccttgggcaaggccgaaggccgcgcagtcgatcaacaagccccggaggggccactttttgccggagggggagccgcgccgaaggcgtgggggaaccccgcaggggtgcccttctttgggcaccaaagaactagatatagggcgaaatgcgaaagacttaaaaatcaacaacttaaaaaaggggggtacgcaacagctcattgcggcaccccccgcaatagctcattgcgtaggttaaagaaaatctgtaattgactgccacttttacgcaacgcataattgttgtcgcgctgccgaaaagttgcagctgattgcgcatggtgccgcaaccgtgcggcaccctaccgcatggagataagcatggccacgcagtccagagaaatcggcattcaagccaagaacaagcccggtcactgggtgcaaacggaacgcaaagcgcatgaggcgtgggccgggcttattgcgaggaaacccacggcggcaatgctgctgcatcacctcgtggcgcagatgggccaccagaacgccgtggtggtcagccagaagacactttccaagctcatcggacgttctttgcggacggtccaatacgcagtcaaggacttggtggccgagcgctggatctccgtcgtgaagctcaacggccccggcaccgtgtcggcctacgtggtcaatgaccgcgtggcgtggggccagccccgcgaccagttgcgcctgtcggtgttcagtgccgccgtggtggttgatcacgacgaccaggacgaatcgctgttggggcatggcgacctgcgccgcatcccgaccctgtatccgggcgagcagcaactaccgaccggccccggcgaggagccgcccagccagcccggcattccgggcatggaaccagacctgccagccttgaccgaaacggaggaatgggaacggcgcgggcagcagcgcctgccgatgcccgatgagccgtgttttctggacgatggcgagccgttggagccgccgacacgggtcacgctgccgcgccggtagggcatcaaataaaacgaaaggctcagtcgaaagactgggcctttcgttttatctgttgtttgtcggtgaacgctctcctgagtaggacaaatccgccgccctagagcgcaacgcaattaatgtaagttagcgcgaattgatctggtttgacagcttatcatcgactgcacggtgcaccaatgcttctggcgtcaggcagccatcggaagctgtggtatggctgtgcaggtcgtaaatcactgcataattcgtgtcgctcaaggcgcactcccgttctggataatgttttttgcgccgacatcataacggttctggcaaatattctgaaatgagctgttgacaattaatcatccggctcgtataatgtgtggaattgtgagcggataacaattaggaggaaaaacatatggcaactgaggagatgaagaaattggccaccgtgatggccattggcacggccaaccctccgaactgctactaccaggccgactttcccgacttctacttccgcgtcaccaacagcgaccacctcatcaacctcaagcaaaagttcaagcgcctttgtgaaaactcaaggattgagaagcgttaccttcatgtgaccgaagagattctcaaggaaaacccaaacattgctgcctacgaggcaacctcgttgaatgtaagacacaaaatgcaagtgaaaggagttgcagagcttgggaaagaggctgccctcaaggccatcaaagaatggggccaacccaagtccaagatcacacatctcatcgtgtgttgcctagccggcgttgacatgcccggcgcggattatcaactcactaagcttcttgaccttgacccttccgtcaagcgttttatgttttaccacctaggatgctacgctggtggcactgtccttcgccttgcaaaggacatagcggagaacaacaagggagctcgtgttctcatcgtttgctcagagatgacaacaacttgttttcgtgggccatctgaaacccatctggactccatgataggccaagcaatattaggcgatggggctgcagctgtcatagttggcgcagatccagacctaaccgttgagaggcccatattcgagttggtttccacagcccagactattgtacccgaatcccatggtgcaattgagggccacttgcttgaatctggactcagtttccatttgtacaagaccgttcctacactaatctctaacaacattaaaacttgcctttctgatgctttcgctcctctaaacattagcgattggaactctcttttctggatcgcacaccctggtggtcctgccatcctagaccaagttactgctaaggttggtcttgaaaaggagaaactcaaggtaactagacaagtgttgaaggactatggaaacatgtcgagtgctacggtgtttttcatcatggatgagatgaggaagaagtcactcgaaaacggtcaagcaaccactggagaagggctcgagtggggtgttttgtttgggttcgggcctggaatcaccgttgaaactgtagtgctacgcagtgtgcccgtaattagctagcttggactcctgttgatagatccagtaatgacctcagaactccatctggatttgttcagaacgctcggttgccgccgggcgttttttattggtgagaatccagattgcgttgcgctcactgcccgctttccagtcgggaaacctgtcgtgccagctgcattaatgaatcggccaacgcgcggggagaggcggtttgcgtattgggcgcatgcataaaaactgttgtaattcattaagcattctgccgacatggaagccatcacaaacggcatgatgaacctgaatcgccagcggcatcagcaccttgtcgccttgcgtataatatttgcccatgggggtgggcgaagaactccagcatgagatccccgcgctggaggatcatccagccggcgtcccggaaaacgattccgaagcccaacctttcatagaaggcggcggtggaatcgaaatctcgtgatggcaggttgggcgtcgcttggtcggtcatttcgaaccccagagtcccgctcagaagaactcgtcaagaaggcgatagaaggcgatgcgctgcgaatcgggagcggcgataccgtaaagcacgaggaagcggtcagcccattcgccgccaagctcttcagcaatatcacgggtagccaacgctatgtcctgatagcggtccgccacacccagccggccacagtcgatgaatccagaaaagcggccattttccaccatgatattcggcaagcaggcatcgccatgggtcacgacgagatcctcgccgtcgggcatgcgcgccttgagcctggcgaacagttcggctggcgcgagcccctgatgctcttcgtccagatcatcctgatcgacaagaccggcttccatccgagtacgtgctcgctcgatgcgatgtttcgcttggtggtcgaatgggcaggtagccggatcaagcgtatgcagccgccgcattgcatcagccatgatggatactttctcggcaggagcaaggtgagatgacaggagatcctgccccggcacttcgcccaatagcagccagtcccttcccgcttcagtgacaacgtcgagcacagctgcgcaaggaacgcccgtcgtggccagccacgatagccgcgctgcctcgtcctgcagttcattcagggcaccggacaggtcggtcttgacaaaaagaaccgggcgcccctgcgctgacagccggaacacggcggcatcagagcagccgattgtctgttgtgcccagtcatagccgaatagcctctccacccaagcggccggagaacctgcgtgcaatccatcttgttcaatcatgcgaaacgatcctcatcctgtctcttgatcagatcttgatcccctgcgccatcagatccttggcggcaagaaagccatccagtttactttgcagggcttcccaaccttaccagagggcgccccagctggcaattccggttcgcttgctgtccataaaaccgcccagtctagctatcgccatgtaagcccactgcaagctacctgctttctctttgcgcttgcgttttcccttgtccagatagcccagtagctgacattcatcccaggtggcacttttcggggaaatgtgcgcgcccgcgttcctgctggcgctgggcctgtttctggcgctggacttcccgctgttccgtcagcagcttttcgcccacggccttgatgatcgcggcggccttggcctgcatatcccgattcaacggccccagggcgtccagaacgggcttcaggcgctcccgaaggt

SEQ ID NO: 5 - DNA, 1155 bp, Rheum palmatum
  source 1..1155: mol_type = other DNA
atggcaactgaggagatgaagaaattggccaccgtgatggccattggcacggccaaccctccgaactgctactaccaggccgactttcccgacttctacttccgcgtcaccaacagcgaccacctcatcaacctcaagcaaaagttcaagcgcctttgtgaaaactcaaggattgagaagcgttaccttcatgtgaccgaagagattctcaaggaaaacccaaacattgctgcctacgaggcaacctcgttgaatgtaagacacaaaatgcaagtgaaaggagttgcagagcttgggaaagaggctgccctcaaggccatcaaagaatggggccaacccaagtccaagatcacacatctcatcgtgtgttgcctagccggcgttgacatgcccggcgcggattatcaactcactaagcttcttgaccttgacccttccgtcaagcgttttatgttttaccacctaggatgctacgctggtggcactgtccttcgccttgcaaaggacatagcggagaacaacaagggagctcgtgttctcatcgtttgctcagagatgacaacaacttgttttcgtgggccatctgaaacccatctggactccatgataggccaagcaatattaggcgatggggctgcagctgtcatagttggcgcagatccagacctaaccgttgagaggcccatattcgagttggtttccacagcccagactattgtacccgaatcccatggtgcaattgagggccacttgcttgaatctggactcagtttccatttgtacaagaccgttcctacactaatctctaacaacattaaaacttgcctttctgatgctttcactcctctaaacattagcgattggaactctcttttctggatcgcacaccctggtggtcctgccatcctagaccaagttactgctaaggttggtcttgaaaaggagaaactcaaggtaactagacaagtgttgaaggactatggaaacatgtcgagtgctacggtgtttttcatcatggatgagatgaggaagaagtcactcgaaaacggtcaagcaaccactggagaagggctcgagtggggtgttttgtttgggttcgggcctggaatcaccgttgaaactgtagtgctacgcagtgtgcccgtaattagctag

SEQ ID NO: 6 - DNA, 4620 bp, synthetic construct
  source 1..4620: mol_type = other DNA
ctcgggccgtctcttgggcttgatcggccttcttgcgcatctcacgcgctcctgcggcggcctgtagggcaggctcatacccctgccgaaccgcttttgtcagccggtcggccacggcttccggcgtctcaacgcgctttgagattcccagcttttcggccaatccctgcggtgcataggcgcgtggctcgaccgcttgcgggctgatggtgacgtggcccactggtggccgctccagggcctcgtagaacgcctgaatgcgcgtgtgacgtgccttgctgccctcgatgccccgttgcagccctagatcggccacagcggccgcaaacgtggtctggtcgcgggtcatctgcgctttgttgccgatgaactccttggccgacagcctgccgtcctgcgtcagcggcaccacgaacgcggtcatgtgcgggctggtttcgtcacggtggatgctggccgtcacgatgcgatccgccccgtacttgtccgccagccacttgtgcgccttctcgaagaacgccgcctgctgttcttggctggccgacttccaccattccgggctggccgtcatgacgtactcgaccgccaacacagcgtccttgcgccgcttctctggcagcaactcgcgcagtcggcccatcgcttcatcggtgctgctggccgcccagtgctcgttctctggcgtcctgctggcgtcagcgttgggcgtctcgcgctcgcggtaggcgtgcttgagactggccgccacgttgcccattttcgccagcttcttgcatcgcatgatcgcgtatgccgccatgcctgcccctcccttttggtgtccaaccggctcgacgggggcagcgcaaggcggtgcctccggcgggccactcaatgcttgagtatactcactagactttgcttcgcaaagtcgtgaccgcctacggcggctgcggcgccctacgggcttgctctccgggcttcgccctgcgcggtcgctgcgctcccttgccagcccgtggatatgtggacgatggccgcgagcggccaccggctggctcgcttcgctcggcccgtggacaaccctgctggacaagctgatggacaggctgcgcctgcccacgagcttgaccacagggattgcccaccggctacccagccttcgaccacatacccaccggctccaactgcgcggcctgcggccttgccccatcaatttttttaattttctctggggaaaagcctccggcctgcggcctgcgcgcttcgcttgccggttggacaccaagtggaaggcgggtcaaggctcgcgcagcgaccgcgcagcggcttggccttgacgcgcctggaacgacccaagcctatgcgagtgggggcagtcgaaggcgaagcccgcccgcctgccccccgagcctcacggcggcgagtgcgggggttccaagggggcagcgccaccttgggcaaggccgaaggccgcgcagtcgatcaacaagccccggaggggccactttttgccggagggggagccgcgccgaaggcgtgggggaaccccgcaggggtgcccttctttgggcaccaaagaactagatatagggcgaaatgcgaaagacttaaaaatcaacaacttaaaaaaggggggtacgcaacagctcattgcggcaccccccgcaatagctcattgcgtaggttaaagaaaatctgtaattgactgccacttttacgcaacgcataattgttgtcgcgctgccgaaaagttgcagctgattgcgcatggtgccgcaaccgtgcggcaccctaccgcatggagataagcatggccacgcagtccagagaaatcggcattcaagccaagaacaagcccggtcactgggtgcaaacggaacgcaaagcgcatgaggcgtgggccgggcttattgcgaggaaacccacggcggcaatgctgctgcatcacctcgtggcgcagatgggccaccagaacgccgtggtggtcagccagaagacactttccaagctcatcggacgttctttgcggacggtccaatacgcagtcaaggacttggtggccgagcgctggatctccgtcgtgaagctcaacggccccggcaccgtgtcggcctacgtggtcaatgaccgcgtggcgtggggccagccccgcgaccagttgcgcctgtcggtgttcagtgccgccgtggtggttgatcacgacgaccaggacgaatcgctgttggggcatggcgacctgcgccgcatcccgaccctgtatccgggcgagcagcaactaccgaccggccccggcgaggagccgcccagccagcccggcattccgggcatggaaccagacctgccagccttgaccgaaacggaggaatgggaacggcgcgggcagcagcgcctgccgatgcccgatgagccgtgttttctggacgatggcgagccgttggagccgccgacacgggtcacgctgccgcgccggtagggcatcaaataaaacgaaaggctcagtcgaaagactgggcctttcgttttatctgttgtttgtcggtgaacgctctcctgagtaggacaaatccgccgccctagagcgcaacgcaattaatgtaagttagcgcgaattgatctggtttgacagcttatcatcgactgcacggtgcaccaatgcttctggcgtcaggcagccatcggaagctgtggtatggctgtgcaggtcgtaaatcactgcataattcgtgtcgctcaaggcgcactcccgttctggataatgttttttgcgccgacatcataacggttctggcaaatattctgaaatgagctgttgacaattaatcatccggctcgtataatgtgtggaattgtgagcggataacaattaggaggaaaaacatcttggactcctgttgatagatccagtaatgacctcagaactccatctggatttgttcagaacgctcggttgccgccgggcgttttttattggtgagaatccagattgcgttgcgctcactgcccgctttccagtcgggaaacctgtcgtgccagctgcattaatgaatcggccaacgcgcggggagaggcggtttgcgtattgggcgcatgcataaaaactgttgtaattcattaagcattctgccgacatggaagccatcacaaacggcatgatgaacctgaatcgccagcggcatcagcaccttgtcgccttgcgtataatatttgcccatgggggtgggcgaagaactccagcatgagatccccgcgctggaggatcatccagccggcgtcccggaaaacgattccgaagcccaacctttcatagaaggcggcggtggaatcgaaatctcgtgatggcaggttgggcgtcgcttggtcggtcatttcgaaccccagagtcccgctcagaagaactcgtcaagaaggcgatagaaggcgatgcgctgcgaatcgggagcggcgataccgtaaagcacgaggaagcggtcagcccattcgccgccaagctcttcagcaatatcacgggtagccaacgctatgtcctgatagcggtccgccacacccagccggccacagtcgatgaatccagaaaagcggccattttccaccatgatattcggcaagcaggcatcgccatgggtcacgacgagatcctcgccgtcgggcatgcgcgccttgagcctggcgaacagttcggctggcgcgagcccctgatgctcttcgtccagatcatcctgatcgacaagaccggcttccatccgagtacgtgctcgctcgatgcgatgtttcgcttggtggtcgaatgggcaggtagccggatcaagcgtatgcagccgccgcattgcatcagccatgatggatactttctcggcaggagcaaggtgagatgacaggagatcctgccccggcacttcgcccaatagcagccagtcccttcccgcttcagtgacaacgtcgagcacagctgcgcaaggaacgcccgtcgtggccagccacgatagccgcgctgcctcgtcctgcagttcattcagggcaccggacaggtcggtcttgacaaaaagaaccgggcgcccctgcgctgacagccggaacacggcggcatcagagcagccgattgtctgttgtgcccagtcatagccgaatagcctctccacccaagcggccggagaacctgcgtgcaatccatcttgttcaatcatgcgaaacgatcctcatcctgtctcttgatcagatcttgatcccctgcgccatcagatccttggcggcaagaaagccatccagtttactttgcagggcttcccaaccttaccagagggcgccccagctggcaattccggttcgcttgctgtccataaaaccgcccagtctagctatcgccatgtaagcccactgcaagctacctgctttctctttgcgcttgcgttttcccttgtccagatagcccagtagctgacattcatcccaggtggcacttttcggggaaatgtgcgcgcccgcgttcctgctggcgctgggcctgtttctggcgctggacttcccgctgttccgtcagcagcttttcgcccacggccttgatgatcgcggcggccttggcctgcatatcccgattcaacggccccagggcgtccagaacgggcttcaggcgctcccgaaggt

SEQ ID NO: 7 - protein, 384 aa, synthetic construct
MATEEMKKLATVMAIGTANPPNCYYQADFPDFYFRVTNSDHLINLKQKFKRLCENSRIEKRYLHVTEEILKENPNIAAYEATSLNVRHKMQVKGVAELGKEAALKAIKEWGQPKSKITHLIVCCLAGVDMPGADYQLTKLLDLDPSVKRFMFYHLGCYAGGTVLRLAKDIAENNKGARVLIVCSEMTTTCFRGPSETHLDSMIGQAILGDGAAAVIVGADPDLTVERPIFELVSTAQTIVPESHGAIEGHLLESGLSFHLYKTVPTLISNNIKTCLSDAFLPLNISDWNSLFWIAHPGGPAILDQVTAKVGLEKEKLKVTRQVLKDYGNMSSATVFFIMDEMRKKSLENGQATTGEGLEWGVLFGFGPGITVETVVLRSVPVIS

SEQ ID NO: 8 - protein, 384 aa, synthetic construct
MATEEMKKLATVMAIGTANPPNCYYQADFPDFYFRVTNSDHLINLKQKFKRLCENSRIEKRYLHVTEEILKENPNIAAYEATSLNVRHKMQVKGVAELGKEAALKAIKEWGQPKSKITHLIVCCLAGVDMPGADYQLTKLLDLDPSVKRFMFYHLGCYAGGTVLRLAKDIAENNKGARVLIVCSEMTTTCFRGPSETHLDSMIGQAILGDGAAAVIVGADPDLTVERPIFELVSTAQTIVPESHGAIEGHLLESGLSFHLYKTVPTLISNNIKTCLSDAFIPLNISDWNSLFWIAHPGGPAILDQVTAKVGLEKEKLKVTRQVLKDYGNMSSATVFFIMDEMRKKSLENGQATTGEGLEWGVLFGFGPGITVETVVLRSVPVIS

SEQ ID NO: 9 - protein, 384 aa, synthetic construct
MATEEMKKLATVMAIGTANPPNCYYQADFPDFYFRVTNSDHLINLKQKFKRLCENSRIEKRYLHVTEEILKENPNIAAYEATSLNVRHKMQVKGVAELGKEAALNAIKEWGQPKSKITHLIVCCLAGVDMPGADYQLTKLLDLDPSVKRFMFYHLGCYAGGTVLRLAKDIAENNKGARVLIVCSEMTTTCFRGPSETHLDSMIGQAILGDGAAAVIVGADPDLTVERPIFELVSTAQTIVPESHGAIEGHLLESGLSFHLYKTVPTLISNNIKTCLSDAFIPLNISDWNSLFWIAHPGGPAILDQVTAKVGLEKEKLKVTRQVLKDYGNMSSATVFFIMDEMRKKSLENGQATTGEGLEWGVLFGFGPGITVETVVLRSVPVIS

SEQ ID NO: 10 - protein, 384 aa, synthetic construct
MATEEMKKLATVMAIGTANPPNCYYQADFPDFYFRVTNSDHLINLKQKFKRLCENSRIEKRYLHVTEEILKENPNIAAYEATSLNVRHKMQVKGVAELGKEAALKAIKEWDQPKSKITHLIVCCLAGVDMPGADYQLTKLLDLDPSVKRFMFYHLGCYAGGTVLRLAKDIAENNKGARVLIVCSEMTTTCFRGPSETHLDSMIGQAILGDGAAAVIVGADPDLTVERPIFELVSTAQTIVPESHGAIEGHLLESGLSFHLYKTVPTLISNNIKTCLSDAFIPLNISDWNSLFWIAHPGGPAILDQVTAKVGLEKEKLKVTRQVLKDYGNMSSATVFFIMDEMRKKSLENGQATTGEGLEWGVLFGFGPGITVETVVLRSVPVIS

SEQ ID NO: 11 - protein, 384 aa, synthetic construct
MATEEMKKLATVMAIGTANPPNCYYQADFPDFYFRVTNSDHLINLKQKFKRLCENSRIEKRYLHVTEEILKENPNIAAYEATSLNVRHKMQVKGVAELGKEAALKAIKEWGQPKSKITHLIVCCLAGVDMPGADYQLTKLLDLDPSVKRFMFYHLGCYAGGTVLRLAKDIAENNKGARVLIVCSEMTTTCFRGPSETHLDSMIGQAILGDGAAAVIVGADPDLTVERPIFELVSTAQTIVPESHGAIEGHLLESGLSFHLYKTVPTLISNNIKTCLSDAFCPLNISDWNSLFWIAHPGGPAILDQVTAKVGLEKEKLKVTRQVLKDYGNMSSATVFFIMDEMRKKSLENGQATTGEGLEWGVLFGFGPGITVETVVLRSVPVIS

SEQ ID NO: 12 - protein, 384 aa, synthetic construct
MATEEMKKLATVMAIGTANPPNCYYQADFPDFYFRVTNSDHLINLKQKFKRLCENSRIEKRYLHVTEEILKENPNIAAYEATSLNVRHKMQVKGVAELGKEAALKAIKEWGQPKSKITHLIVCCLAGVDMPGADYQLTKLLDLDPSVKRFMFYHLGCYAGGTVLRLAKDIAENNKGARVLIVCSEMTTTCFRGPSETHLDSMIGQAILGDGAAAVIVGADPDLTVERPIFELVSTAQTIVPESHGAIEGHLLESGLSFHLYKTVPTLISNNIKTCLSDAFKPLNISDWNSLFWIAHPGGPAILDQVTAKVGLEKEKLKVTRQVLKDYGNMSSATVFFIMDEMRKKSLENGQATTGEGLEWGVLFGFGPGITVETVVLRSVPVIS

SEQ ID NO: 13 - protein, 384 aa, synthetic construct
MATEEMKKLATVMAIGTANPPNCYYQADFPDFYFRVTNSDHLINLKQKFKRLCENSRIEKRYLHVTEEILKENPNIAAYEATSLNVRHKMQVKGVAELGKEAALKAIKEWGQPKSKITHLIVCCLAGVDMPGADYQLTKLLDLDPSVKRFMFYHLGCYAGGTVLRLAKDIAENNKGARVLIVCSEMTTTCFRGPSETHLDSMIGQAILGDGAAAVIVGADPDLTVERPIFELVSTAQTIVPESHGAIEGHLLESGLSFHLYKTIPTLISNNIKTCLSDAFKPLNISDWNSLFWIAHPGGPAILDQVTAKVGLEKEKLKVTRQVLKDYGNMSSATVFFIMDEMRKKSLENGQATTGEGLEWGVLFGFGPGITVETVVLRSVPVIS

SEQ ID NO: 14 - protein, 384 aa, synthetic construct
MATEEMKKLATVMAIGTANPPNCYYQADFPDFYFRVTNSDHLINLKQKFKRLCENSRIEKRYLHVTEEILKENPNIAAYEATSLNVRHKMQVKGVAELGKEAALKAIKEWGQPKSKITHLIVCCLAGVDMPGADYQLTKLIDLDPSVKRFMFYHLGCYAGGTVLRLAKDIAENNKGARVLIVCSEMTTTCFRGPSETHLDSMIGQAILGDGAAAVIVGADPDLTVERPIFELVSTAQTIVPESHGAIEGHLLESGLSFHLYKTVPTLISNNIKTCLSDAFTPLNISDWNSLFWIAHPGGPAILDQVTAKVGLEKEKLKVTRQVLKDYGNMSSATVFFIMDEMRKKSLENGQATTGEGLEWGVLFGFGPGITVETVVLRSVPVIS

SEQ ID NO: 15 - protein, 384 aa, synthetic construct
MATEEMKKLATVMAIGTANPPNCYYQADFPDFYFRVTNSDHLINLKQKFKRLCENSRIEKRYLHVTEEILKENPNIAAYEATSLNVRHKMQVKGVAELGKEAALKAIKEWGQPKSKITHLIVCCLAGVDMPGADYQLTKLIDLDPSVKRFMFYHLGCYAGGTVLRLAKDIAENNKGARVLIVCSEMTTTCFRGPSETHLDSMIGQAILGDGAAAVIVGADPDLTVERPIFELVSTAQTIVPESHGAIEGHLLESGLSFHLYKTVPTLISNNIKTCLSDAFAPLNISDWNSLFWIAHPGGPAILDQVTAKVGLEKEKLKVTRQVLKDYGNMSSATVFFIMDEMRKKSLENGQATTGEGLEWGVLFGFGPGITVETVVLRSVPVIS

SEQ ID NO: 16 - protein, 384 aa, synthetic construct
MATEEMKKLATVMAIGTANPPNCYYQADFPDFYFRVTNSDHLINLKQKFKKLCENSRIEKRYLHVTEEILKENPNIAAYEATSLNVRHKMQVKGVAELGKEAALKAIKEWGQPKSKITHLIVCCLAGVDMPGADYQLTKLLDLDPSVKRFMFYHLGCYAGGTVLRLAKDIAENNKGARVLIVCSEMTTTCFRGPSETHLDSMIGQAILGDGAAAVIVGADPDLTVERPIFELVSTAQTIVPESHGAIEGHLLESGLSFHLYKTVPTLISNNIKTCLSDAFTPLNISDWNSLFWIAHPGGPAILDQVTAKVGLEKEKLKVTRQVLKDYGNMSSATVFFIMDEMRKKSLENGQATTGEGLEWGVLFGFGPGITVETVVLRSVPVIS

SEQ ID NO: 17 - protein, 384 aa, synthetic construct
MATEEMKKLATVMAIGTANPPNCYYQADFPDFYFRVTNSDHLINLKQKFKRLCENSRIEKRYLHVTEEILKENPNIAAYEATSLDVRHKMQVKGVAELGKEAALKAIKEWGQPKSKITHLIVCCLAGVDMPGADYQLTKLLDLDPSVKRFMFYHLGCYAGGTVLRLAKDIAENNKGARVLIVCSEMTTTCFRGPSETHLDSMIGQAILGDGAAAVIVGADPDLTVERPIFELVSTAQTIVPESHGAIEGHLLESGLSFHLYKTVPTLISNNIKTCLSDAFTPLNISDWNSLFWIAHPGGPAILDQVTAKVGLEKEKLKVTRQVLKDYGNMSSATVFFIMDEMRKKSLENGQATTGEGLEWGVLFGFGPGITVETVVLRSVPVIS

SEQ ID NO: 18 - protein, 384 aa, synthetic construct
MATEEMKKLATVMAIGTANPPNCYYQADFPDFYFRVTNSDHLINLKQKFKRLCENSRIEKRYLHVTEEILKENPNIAAYEATSLNVRHKMQVKGVAELGKEAALKAIKEWGQPKSKITHLIVCCLAGVDMPGADYQLTKLLDLDPSVKRFMFYHLGCYAGGTVLRLAKDIAENNKGARVLIVCSENTTTCFRGPSETHLDSMIGQAILGDGAAAVIVGADPDLTVERPIFELVSTAQTIVPESHGAIEGHLLESGLSFHLYKTVPTLISNNIKTCLSDAFTPLNISDWNSLFWIAHPGGPAILDQVTAKVGLEKEKLKVTRQVLKDYGNMSSATVFFIMDEMRKKSLENGQATTGEGLEWGVLFGFGPGITVETVVLRSVPVIS

SEQ ID NO: 19 - protein, 384 aa, synthetic construct
MATEEMKKLATVMAIGTANPPNCYYQADFPDFYFRVTNSDHLINLKQKFKRLCENSRIEKRYLHVTEEILKENPNIAAYEATSLNVRHKMQVKGVAELGKEAALKAIKEWGQPKSKITHLIVCCLAGVDMPGADYQLTKLLDLDPSVKRFMFYHLGCYAGGTVLRLAKDIAENNKGARVLIVCSEVTTTCFRGPSETHLDSMIGQAILGDGAAAVIVGADPDLTVERPIFELVSTAQTIVPESHGAIEGHLLESGLSFHLYKTVPTLISNNIKTCLSDAFTPLNISDWNSLFWIAHPGGPAILDQVTAKVGLEKEKLKVTRQVLKDYGNMSSATVFFIMDEMRKKSLENGQATTGEGLEWGVLFGFGPGITVETVVLRSVPVIS

SEQ ID NO: 20 - protein, 384 aa, synthetic construct
MATEEMKKLATVMAIGTANPPNCYYQADFPDFYFRVTNSDHLINLKQKFKRLCENSRIEKRYLHVTEEILKENPNIAAYEATSLNVRHKMQVKGVAELGKEAALKAIKEWGQPKSKITHLIVCCLAGVDMPGADYQLTKLLDLDPSVKRFMFYHLGCYAGGTVLRLAKDIAENNKGARVLIVCSEMTTCCFRGPSETHLDSMIGQAILGDGAAAVIVGADPDLTVERPIFELVSTAQTIVPESHGAIEGHLLESGLSFHLYKTVPTLISNNIKTCLSDAFTPLNISDWNSLFWIAHPGGPAILDQVTAKVGLEKEKLKVTRQVLKDYGNMSSATVFFIMDEMRKKSLENGQATTGEGLEWGVLFGFGPGITVETVVLRSVPVIS

SEQ ID NO: 21 - protein, 384 aa, synthetic construct
MATEEMKKLATVMAIGTANPPNCYYQADFPDFYFRVTNSDHLINLKQKFKRLCENSRIEKRYLHVTEEILKENPNIAAYEATSLNVRHKMQVKGVAELGKEAALKAIKEWGQPKSKITHLIVCCLAGVDMPGADYQLTKLLDLDPSVKRFMFYHLGCYAGGTVLRLAKDIAENNKGARVLIVCSEMTTICFRGPSETHLDSMIGQAILGDGAAAVIVGADPDLTVERPIFELVSTAQTIVPESHGAIEGHLLESGLSFHLYKTVPTLISNNIKTCLSDAFTPLNISDWNSLFWIAHPGGPAILDQVTAKVGLEKEKLKVTRQVLKDYGNMSSATVFFIMDEMRKKSLENGQATTGEGLEWGVLFGFGPGITVETVVLRSVPVIS

SEQ ID NO: 22 - protein, 384 aa, synthetic construct
MATEEMKKLATVMAIGTANPPNCYYQADFPDFYFRVTNSDHLINLKQKFKRLCENSRIEKRYLHVTEEILKENPNIAAYEATSLNVRHKMQVKGVAELGKEAALKAIKEWGQPKSKITHLIVCCLAGVDMPGADYQLTKLLDLDPSVKRFMFYHLGCYAGGTVLRLAKDIAENNKGARVLIVCSEMTTVCFRGPSETHLDSMIGQAILGDGAAAVIVGADPDLTVERPIFELVSTAQTIVPESHGAIEGHLLESGLSFHLYKTVPTLISNNIKTCLSDAFTPLNISDWNSLFWIAHPGGPAILDQVTAKVGLEKEKLKVTRQVLKDYGNMSSATVFFIMDEMRKKSLENGQATTGEGLEWGVLFGFGPGITVETVVLRSVPVIS

SEQ ID NO: 23 - protein, 384 aa, synthetic construct
MATEEMKKLATVMAIGTANPPNCYYQADFPDFYFRVTNSDHLINLKQKFKRLCENSRIEKRYLHVTEEILKENPNIAAYEATSLNVRHKMQVKGVAELGKEAALKAIKEWGQPKSKITHLIVCCLAGVDMPGADYQLTKLLDLDPSVKRFMFYHLGCYAGGTVLRLAKDIAENNKGARVLIVCSEMTTTCFRGPSETHLDSMIGQAILADGAAAVIVGADPDLTVERPIFELVSTAQTIVPESHGAIEGHLLESGLSFHLYKTVPTLISNNIKTCLSDAFTPLNISDWNSLFWIAHPGGPAILDQVTAKVGLEKEKLKVTRQVLKDYGNMSSATVFFIMDEMRKKSLENGQATTGEGLEWGVLFGFGPGITVETVVLRSVPVIS

SEQ ID NO: 24 - protein, 384 aa, synthetic construct
MATEEMKKLATVMAIGTANPPNCYYQADFPDFYFRVTNSDHLINLKQKFKRLCENSRIEKRYLHVTEEILKENPNIAAYEATSLNVRHKMQVKGVAELGKEAALKAIKEWGQPKSKITHLIVCCLAGVDMPGADYQLTKLLDLDPSVKRFMFYHLGCYAGGTVLRLAKDIAENNKGARVLIVCSEMTTTCFRGPSETHLDSMIGQAILSDGAAAVIVGADPDLTVERPIFELVSTAQTIVPESHGAIEGHLLESGLSFHLYKTVPTLISNNIKTCLSDAFTPLNISDWNSLFWIAHPGGPAILDQVTAKVGLEKEKLKVTRQVLKDYGNMSSATVFFIMDEMRKKSLENGQATTGEGLEWGVLFGFGPGITVETVVLRSVPVIS

SEQ ID NO: 25 - protein, 384 aa, synthetic construct
MATEEMKKLATVMAIGTANPPNCYYQADFPDFYFRVTNSDHLINLKQKFKRLCENSRIEKRYLHVTEEILKENPNIAAYEATSLNVRHKMQVKGVAELGKEAALKAIKEWGQPKSKITHLIVCCLAGVDMPGADYQLTKLLDLDPSVKRFMFYHLGCYAGGTVLRLAKDIAENNKGARVLIVCSEMTTTCFRGPSETHLDSMIGQAILGDGAAAVIVGADPDLTVERPIFELVSTAQTIVPESHGAIEGHLLESGLSFHLYKTVPTLIANNIKTCLSDAFTPLNISDWNSLFWIAHPGGPAILDQVTAKVGLEKEKLKVTRQVLKDYGNMSSATVFFIMDEMRKKSLENGQATTGEGLEWGVLFGFGPGITVETVVLRSVPVIS

SEQ ID NO: 26 - protein, 384 aa, synthetic construct
MATEEMKKLATVMAIGTANPPNCYYQADFPDFYFRVTNSDHLINLKQKFKRLCENSRIEKRYLHVTEEILKENPNIAAYEATSLNVRHKMQVKGVAELGKEAALKAIKEWGQPKSKITHLIVCCLAGVDMPGADYQLTKLLDLDPSVKRFMFYHLGCYAGGTVLRLAKDIAENNKGARVLIVCSEMTTTCFRGPSETHLDSMIGQAILGDGAAAVIVGADPDLTVERPIFELVSTAQTIVPESHGAIEGHLLESGLSFHLYKTVPTLISNNIKTCLSDAFTPLNISDWNSLFWIVHPGGPAILDQVTAKVGLEKEKLKVTRQVLKDYGNMSSATVFFIMDEMRKKSLENGQATTGEGLEWGVLFGFGPGITVETVVLRSVPVIS

SEQ ID NO: 27 - protein, 384 aa, synthetic construct
MATEEMKKLATVMAIGTANPPNCYYQADFPDFYFRVTNSDHLINLKQKFKRLCENSRIEKRYLHVTEEILKENPNIAAYEATSLNVRHKMQVKGVAELGKEAALKAIKEWGQPKSKITHLIVCCLAGVDMPGADYQLTKLLDLDPSVKRFMFYHLGCYAGGTVLRLAKDIAENNKGARVLIVCSEMTTTCFRGPSETHLDSMIGQAILGDGAAAVIVGADPDLTVERPIFELVSTAQTIVPESHGAIEGHLLESGLSFHLYKTIPTLISNNIKTCLSDAFTPLNISDWNSLFWIAHPGGPAILDQVTAKVGLEKEKLKVTRQVLKDYGNMSSATVFFIMDEMRKKSLENGQATTGEGLEWGVLFGFGPGITVETVVLRSVPVIS

SEQ ID NO: 28 - protein, 384 aa, synthetic construct
MATEEMKKLATVMAIGTANPPNCYYQADFPDFYFRVTNSDHLINLKQKFKRLCENSRIEKRYLHVTEEILKENPNIAAYEATSLNVRHKMQVKGVAELGKEAALKAIKEWGQPKSKITHLIVCCLAGVDMPGADYQLTKLIDLDPSVKRFMFYHLGCYAGGTVLRLAKDIAENNKGARVLIVCSEMTTTCFRGPSETHLDSMIGQAILGDGAAAVIVGADPDLTVERPIFELVSTAQTIVPESHGAIEGHLLESGLSFHLYKTIPTLISNNIKTCLSDAFTPLNISDWNSLFWIAHPGGPAILDQVTAKVGLEKEKLKVTRQVLKDYGNMSSATVFFIMDEMRKKSLENGQATTGEGLEWGVLFGFGPGITVETVVLRSVPVIS

SEQ ID NO: 29 - protein, 384 aa, synthetic construct
MATEEMKKLATVMAIGTANPPNCYYQADFPDFYFRVTNSDHLINLKQKFKRLCENSRIEKRYLHVTEEILKENPNIAAYEATSLNVRHKMQVKGVAELGKEAALKAIKEWGQPKSKITHLIVCCLAGVDMPGADYQLTKLIDLDPSVKRFMFYHLGCYAGGTVLRLAKDIAENNKGARVLIVCSEMTTTCFRGPSETHLDSMIGQAILGDGAAAVIVGADPDLTVERPIFELVSTAQTIVPESHGAIEGHLLESGLSFHLYKTIPTLISNNIKTCLSDAFAPLNISDWNSLFWIAHPGGPAILDQVTAKVGLEKEKLKVTRQVLKDYGNMSSATVFFIMDEMRKKSLENGQATTGEGLEWGVLFGFGPGITVETVVLRSVPVIS